European Patent Application EP 4 112 646 A1, published January 4, 2023. Title: MONOCLONAL ANTIBODY OF MATRIX METALLOPROTEINASE-1, DETECTION KIT AND DETECTION METHOD THEREOF. Applicant: S&T BIOMED CO., LTD. Application EP20921555.7. The sequence listing filed with the application follows.

SEQUENCE LISTING (18 sequences)

SEQ ID NO: 1 - protein, 10 aa, Artificial Sequence
  V_segment: CDR1 of heavy chain variable region sequence of monoclonal antibody 31-34
GYSFTDYIML

SEQ ID NO: 2 - protein, 17 aa, Artificial Sequence
  V_segment: CDR2 of heavy chain variable region sequence of monoclonal antibody 31-34
NINPHYGGTSYNLKFKG

SEQ ID NO: 3 - protein, 11 aa, Artificial Sequence
  V_segment: CDR3 of heavy chain variable region sequence of monoclonal antibody 31-34
ARYGFSAWFAY

SEQ ID NO: 4 - protein, 11 aa, Artificial Sequence
  V_segment: CDR1 of light chain variable region sequence of monoclonal antibody 31-34
RASENIYSNLA

SEQ ID NO: 5 - protein, 7 aa, Artificial Sequence
  V_segment: CDR2 of light chain variable region sequence of monoclonal antibody 31-34
AATNLAD

SEQ ID NO: 6 - protein, 9 aa, Artificial Sequence
  V_segment: CDR3 of light chain variable region sequence of monoclonal antibody 31-34
QHFWGIPFT

SEQ ID NO: 7 - protein, 7 aa, Artificial Sequence
  V_segment: CDR1 of heavy chain variable region sequence of monoclonal antibody 73-1
GYTFSNY

SEQ ID NO: 8 - protein, 17 aa, Artificial Sequence
  V_segment: CDR2 of heavy chain variable region sequence of monoclonal antibody 73-1
EILPGGGNTYHNEKFKG

SEQ ID NO: 9 - protein, 13 aa, Artificial Sequence
  V_segment: CDR3 of heavy chain variable region sequence of monoclonal antibody 73-1
ARSGDDYDDVFAY

SEQ ID NO: 10 - protein, 15 aa, Artificial Sequence
  V_segment: CDR1 of light chain variable region sequence of monoclonal antibody 73-1
RASESVDSHGKTFMH

SEQ ID NO: 11 - protein, 7 aa, Artificial Sequence
  V_segment: CDR2 of light chain variable region sequence of monoclonal antibody 73-1
RASNLES

SEQ ID NO: 12 - protein, 9 aa, Artificial Sequence
  V_segment: CDR3 of light chain variable region sequence of monoclonal antibody 73-1
QQSNEDPWT

SEQ ID NO: 13 - protein, 7 aa, Artificial Sequence
  V_segment: CDR1 of heavy chain variable region sequence of monoclonal antibody 1-8A12
GYTFTNY

SEQ ID NO: 14 - protein, 17 aa, Artificial Sequence
  V_segment: CDR2 of heavy chain variable region sequence of monoclonal antibody 1-8A12
DIYPYSGTTNYNEKFKS

SEQ ID NO: 15 - protein, 12 aa, Artificial Sequence
  V_segment: CDR3 of heavy chain variable region sequence of monoclonal antibody 1-8A1
ARDEITSPYFSY

SEQ ID NO: 16 - protein, 11 aa, Artificial Sequence
  V_segment: CDR1 of light chain variable region sequence of monoclonal antibody 1-8A12
KASQSVGHDVA

SEQ ID NO: 17 - protein, 7 aa, Artificial Sequence
  V_segment: CDR2 of light chain variable region sequence of monoclonal antibody 1-8A12
YASNRYT

SEQ ID NO: 18 - protein, 9 aa, Artificial Sequence
  V_segment: CDR3 of light chain variable region sequence of monoclonal antibody 1-8A12
QQDYSSPWT